European Patent Specification EP 4 408 858 B1, published March 11, 2026. Title: RECOMBINANT GLYCAN BINDING PROTEINS AND ITS USE. Applicant: Unichem Laboratories Limited. Application IN. The sequence listing filed with the application follows.

SEQUENCE LISTING (6 sequences)

SEQ ID NO: 1 - protein, 141 aa, synthetic construct
TYKITVRVYQTNPNAFFHPVEKTVWKYANGGTWTITDDQHVLTMGGSGTSGTLRFHADNGESFTATFGVHNYKRWCDIVTNLAADETGMVINQQYYSQKNREEARERQLSNYEVKNAKGRNFEIVYTEAEGNDLHANLIIG

SEQ ID NO: 2 - protein, 141 aa, synthetic construct
TYKITVRVYQTNPDAFFHPVEKTVWKYANGGTWTITDDQHVLTMGGSGTSGTLRFHADNGESFTATFGVHNYKRWCDIVTNLAADETGMVINQQYYSQKNREEARERQLSNYQVKNAKGRNFQIVYTEAEGNDLHANLIIG

SEQ ID NO: 3 - protein, 142 aa, synthetic construct
SYKITVRVYQTNPDAFFHPVEKTVWKYANGGTWTITDDQHVLTMGGSGTSGTLRFHADNGESFTATFGVHNYKRWGDIVTNLAADETGMVINQQYYSQKNREEARERQLSNYQVKNAKGRNFQIVYTEAEGNDLHANLIIGC

SEQ ID NO: 4 - protein, 143 aa, synthetic construct
SYKITVRVYQTNPDAFFHPVEKTVWKYANGGTWTITDDQHVLTMGGSGTSGTLRFHADNGESFTATFGVHNYKRWGDIVTNLAADETGMVINQQYYSQKNREEARERQLSNYQVKNAKGRNFQIVYTEAEGNDLHANLIIGSC

SEQ ID NO: 5 - DNA, 426 bp, synthetic construct
  source 1..426: mol_type = other DNA
agctataaaattaccgtgcgcgtgtatcagaccaacccggatgcctttttccatccggtggaaaaaaccgtgtggaaatatgcgaatggcggtacctggacgattacggatgatcagcatgtgctgacgatgggtggtagcggtaccagcggcaccctgcgttttcacgcagataatggcgaaagcttcaccgccacctttggtgtgcataattataaacgctggggcgatattgtgaccaacctggcagcggatgaaaccggcatggttattaatcagcagtattatagtcagaaaaaccgcgaagaagcgcgtgaacgccagctgagtaactatcaggtgaaaaatgcgaaaggccgtaacttccagattgtttataccgaagcggaaggcaatgatctgcatgcgaacctgattatcggctgc

SEQ ID NO: 6 - DNA, 429 bp, synthetic construct
  source 1..429: mol_type = other DNA
agctataaaattaccgtgcgcgtgtatcagaccaacccggatgcctttttccatccggtggaaaaaaccgtgtggaaatatgcgaatggcggtacctggacgattacggatgatcagcatgtgctgacgatgggtggtagcggtaccagcggcaccctgcgttttcacgcagataatggcgaaagcttcaccgccacctttggtgtgcataattataaacgctggggcgatattgtgaccaacctggcagcggatgaaaccggcatggttattaatcagcagtattatagtcagaaaaaccgcgaagaagcgcgtgaacgccagctgagtaactatcaggtgaaaaatgcgaaaggccgtaacttccagattgtttataccgaagcggaaggcaatgatctgcatgcgaacctgattatcggcagctgc